European Patent Specification EP 4 217 007 B1, published November 6, 2024. Title: Peptidic conjugates of SN38 useful in the treatment of cancer. Applicant: FUNDACIO INSTITUT DE RECERCA BIOMEDICA (IRB BARCELONA) UNIVERSITAT DE BARCELONA HOSPITAL DE SANT JOAN DE DEU. The sequence listing filed with the application follows.

SEQUENCE LISTING (14 sequences)

SEQ ID NO: 1 - protein, 9 aa, Artificial Sequence
  PEPTIDE
  misc_feature (1)..(1): Xaa is selected from the group consisting of Dpr and Dbu,  and it is bound to amino acid at position 9 through an amide intrapeptide bond
  misc_feature (9)..(9): Xaa is selected from the group consisting of Asp and Glu,  and it is bound to amino acid at position 1 through an amide intrapeptide bond
XKAPETALX

SEQ ID NO: 2 - protein, 12 aa, Artificial Sequence
  PEPTIDE
  misc_feature (1)..(1): Xaa is an amino acid which is the same as the amino acid at position 9 and it is selected from cysteine, selenocysteine, and penicillamine
  misc_feature (1)..(1): it is bound to the amino acid at position 9 by a disulfide or diselenide intrapeptide bond
  misc_feature (9)..(9): Xaa is an amino acid which is the same as the amino acid at position 1 and it is selected from cysteine, selenocysteine, and penicillamine
  misc_feature (9)..(9): it is bound to the amino acid at position 1 by a disulfide or diselenide intrapeptide bond
XKAPETALXAAA

SEQ ID NO: 3 - protein, 9 aa, Artificial Sequence
  PEPTIDE
  misc_feature (1)..(1): Xaa is an amino acid which is the same as the amino acid at position 9 and it is selected from cysteine, selenocysteine, and penicillamine
  misc_feature (1)..(1): it is bound to the amino acid at position 9 by a disulfide or diselenide intrapeptide bond
  misc_feature (9)..(9): Xaa is an amino acid which is the same as the amino acid at position 1 and it is selected from cysteine, selenocysteine, and penicillamine
  misc_feature (9)..(9): it is bound to the amino acid at position 1 by a disulfide or diselenide intrapeptide bond
XKAPETALX

SEQ ID NO: 4 - protein, 10 aa, Artificial Sequence
  PEPTIDE
  misc_feature (1)..(1): Xaa is an amino acid which is the same as the amino acid at position 9 and it is selected from cysteine, selenocysteine, and penicillamine
  misc_feature (1)..(1): it is bound to the amino acid at position 9 by a disulfide or diselenide intrapeptide bond
  misc_feature (9)..(9): Xaa is an amino acid which is the same as the amino acid at position 1 and it is selected from cysteine, selenocysteine, and penicillamine
  misc_feature (9)..(9): it is bound to the amino acid at position 1 by a disulfide or diselenide intrapeptide bond
XKAPETALXA

SEQ ID NO: 5 - protein, 11 aa, Artificial Sequence
  PEPTIDE
  misc_feature (1)..(1): Xaa is an amino acid which is the same as the amino acid at position 9 and it is selected from cysteine, selenocysteine, and penicillamine
  misc_feature (1)..(1): it is bound to the amino acid at position 9 by a disulfide or diselenide intrapeptide bond
  misc_feature (9)..(9): Xaa is an amino acid which is the same as the amino acid at position 1 and it is selected from cysteine, selenocysteine, and penicillamine
  misc_feature (9)..(9): it is bound to the amino acid at position 1 by a disulfide or diselenide intrapeptide bond
XKAPETALXAA

SEQ ID NO: 6 - protein, 16 aa, Artificial Sequence
  PEPTIDE
  misc_feature (1)..(1): Xaa is an amino acid which is the same as the amino acid at position 11, and it is selected from the group consisting of cysteine, selenocysteine, and penicillamine
  misc_feature (1)..(1): it is bound to the amino acid at position 11 by a disulfide or diselenide intrapeptide bond
  misc_feature (3)..(3): Xaa is an amino acid which is the same as the amino acid at position 15, and it is selected from the group consisting of cysteine, selenocysteine, and penicillamine
  misc_feature (3)..(3): it is bound to the amino acid at position 15 by a disulfide or diselenide intrapeptide bond
  misc_feature (11)..(11): Xaa is an amino acid which is the same as the amino acid at position 1 and it is selected from the group consisting of cysteine, selenocysteine, and penicillamine
  misc_feature (11)..(11): it is bound to the amino acid at position 1 by a disulfide or diselenide intrapeptide bond
  misc_feature (15)..(15): Xaa is an amino acid which is the same as the amino acid at position 3, and it is selected from the group consisting of cysteine, selenocysteine, and penicillamine
  misc_feature (15)..(15): it is bound to the amino acid at position 3 by a disulfide or diselenide intrapeptide bond
XNXKAPETALXAAAXH

SEQ ID NO: 7 - protein, 9 aa, Artificial Sequence
  PEPTIDE
  MISC_FEATURE (1)..(1): Xaa is selected from Dpr and Dpu
  MISC_FEATURE (9)..(9): Xaa is selected from Glu and Asp
XKAPETALX

SEQ ID NO: 8 - protein, 9 aa, Artificial Sequence
  PEPTIDE
  misc_feature (1)..(1): Xaa represents Dap, and it is bound to the amino acid at position 9 by an amide intrapeptide bond
XKAPETALD

SEQ ID NO: 9 - protein, 12 aa, Artificial Sequence
  PEPTIDE
  DISULFID (1)..(9)
CKAPETALCAAA

SEQ ID NO: 10 - protein, 9 aa, Artificial Sequence
  PEPTIDE
  DISULFID (1)..(9)
CKAPETALC

SEQ ID NO: 11 - protein, 10 aa, Artificial Sequence
  PEPTIDE
  DISULFID (1)..(9)
CKAPETALCA

SEQ ID NO: 12 - protein, 11 aa, Artificial Sequence
  PEPTIDE
  DISULFID (1)..(9)
CKAPETALCAA

SEQ ID NO: 13 - protein, 16 aa, Artificial Sequence
  PEPTIDE
  DISULFID (1)..(11)
  DISULFID (3)..(15)
CNCKAPETALCAAACH

SEQ ID NO: 14 - protein, 9 aa, Artificial Sequence
  PEPTIDE
  misc_feature (1)..(1): Xaa means Dpr
XKAPETALD